European Patent Application EP 4 545 651 A1, published April 30, 2025. Title: NOVEL BIOMARKERS FOR PROGNOSIS OF COMMUNITY ACQUIRED PNEUMONIA (CAP). Applicant: Charité Universitätsmedizin Berlin. Application EP. The sequence listing filed with the application follows.

SEQUENCE LISTING (18 sequences)

SEQ ID NO: 1 - DNA, 4336 bp, Homo sapiens
  source 1..4336: mol_type = genomic DNA
gaggttgaaggacccaggcgtgtcagccctgctccagacaccttgggcatggaggagagtgtcgtacggccctcagtgtttgtggtggatggacagaccgacatcccattcacgaggctgggacgaagccaccggagacagtcgtgcagtgtggcccgggacggacctgcaggctcctgggagcagctgatacaagagcgaaggtctcacgaggtcaacccagcagcgcatctcacaggggccaactccagcttgaccggcagcggggggccgctgttatgggagactcagctgggcctggccttcctgaggggcctcagctaccacgatggggcccttgtggtcaccaaagctggctactactacatctactccaaggtgcagctgggcggtgtgggctgcccgctgggcctggccagcaccatcacccacggcctctacaagcgcacaccccgctaccccgaggagctggagctgttggtcagccagcagtcaccctgcggacgggccaccagcagctcccgggtctggtgggacagcagcttcctgggtggtgtggtacacctggaggctggggagaaggtggtcgtccgtgtgctggatgaacgcctggttcgactgcgtgatggtacccggtcttacttcggggctttcatggtgtgaaggaaggagcgtggtgcattggacatgggtctgacacgtggagaactcagagggtgcctcaggggaaagaaaactcacgaagcagaggctgggcgtggtggctctcgcctgtaatcccagcactttgggaggccaaggcaggcggatcacctgaggtcaggagttcgagaccagcctggctaacatggcaaaaccccatctctactaaaaatacaaaaattagccggacgtggtggtgcctgcctgtaatccagctactcaggaggctgaggcaggataattttgcttaaacccgggaggcggaggttgcagtgagccgagatcacaccactgcactccaacctgggaaacgcagtgagactgtgcctcaaaaaaaagaaaggaagaaaaaagaaaactcaggaaacagatcttgggggacactccagggaacccaaaactcaaaggcggagagctcagtgggcaccaccaaggcgagatgaagccccagcaggcaccttcagaagacccacgtagactgcagaccctgccacggacaatactaaggacaaaaacccagagacttggggtctgtgggcccccaaacatggggtaaagttgatttgcctgatattcaggaagaaggggtgaggggtgggtatttatgcttttgattcagaagaaagtggggcttgggattccagggacttggctgggggtgggaaacttcatccacttccctactctcatcatgagtacggacagggtgggcgggagactgatcatcgggactcatcatgaagagcccagccccaccccacatactcagatcccacccacagactggtggccacacctcagcctggtcacaaagagttacactcagatacatgagcacggcagcgtgctcataactgtttaacaaccagctgtcctgggagggggacagctttgtaatgtttgccaatttccatggtgtaaatgctaccaccatggctgatttcatcactgccaagcatagacatccctaataggacaccacggatctgtccccggcatccggcccagggcctggcacaaagcatgctctagggaaatgcttgctgattgaaaggaaggaagaatgactctacagtcacacctatggcatcccacaaaatctgtcacatggctgcataatctcagccactctttcacaactatagactcatacacgcgaagtgccagattcatgcacaaccacacaatcacatggaagtcacagacggcatcacagacagtcacagcactgtgtgtatgttataacacaagcacacaaaactcagacagcatcccagctacacagccactcccagaggtgtcaccgtcacacttggtaattaatactcattacattagacacagacagaccaagttatagtcagacctggttacacacatacacacacacaatatcaccatgacaaatacacattacacacacacaacatcacaatgacaaacacacattacacacacaacatcacgatgacaaacacacattacacacacaacatcacgatgacaaacacacattacacacacatcacaatgacaaacacaacattacacacacacaacatcacaatgacacacacatcacacacacatcacaatgacaaacacacaacattacacacatatacacacagcctgagggccctccccagcccagactaacacatctcggggtgaggaccagaccttgttcataaccctgggcctcttaaccactgatctttgaaataaatggcaaatagttgtacctggatctgtctagttcttaggggaacaaactgaagaagggtggagaggaattgtcaggcctaaagagccccacagggaaagggaggagtcggatggggggcaaccatcagcaacaagtggtggctcctagaggcagagggatggaggtaatgacccatggaggtcattctacagatgaggaacctggacccagttggctcaagtccatgcaggaaatgtgggggaaaccagagacctcacgtctggatctggcttcctctccaatccacaattcctgaggaagtagaggctacatcccgcaagacgcccttattagacacatccaggacagaatgacaatccgccaagccagctggaagcataaaacacagggagctggtgggttgggtgggggcagataatgatatgcatacaaattagagggtctatgcaaatgagcattgctgcagtgtggctggagggaatccttagttcctaggattctaggatatgggtttcgaccccagaggtgaatgtattgttattattgttttgttgttgttgtgaatgacaagtcaaaatttgtgggttattgttgttatcgccaatagtattcttgtcattgttgcacagtacagagatgaaggaaacagattttgcaatcagatgatcctgggttctgagtccactctgccactcaccagctatatgacctccagcaatttccatcacctctcaatgcttcagtttccccatcggcaagatggttgtggggggagaggaacaacagtacagattcaccatcccaaattcaaaatgctccaaaatctaggccgggcgtggtggctcatacctgtaatcccagcactttgggaggtcaaagtggacggataacctgaggtcaggagctccagaccagcctggccaacatggcgaaaccccatctctactaaaaatacaaaaaattacctgggtgtggtggggggcacctgtaaccccagctactcgggaggctgaggcaggaaccctggaggttgaggttgcagtgagctgagatcacaccactgcactccagcctgggtgacagagcaaggctcccatctcaaaaaacaaaaaaacatgctccaaaatctgaaactctttgagccccagtgtgatgccacaagtgggaaattccacaactcatcacatgtgatagattgcagtggaaatgcaggcacacaccacgaagtttactcagcatcctcaaaggaaatccccgtcagtagctatatatcattttctcacatgccagataggtatctctcatcttttactgttaggtacttctgtgttgaataggtggaggaaaatgattgctggttagtagtatataaattcagagtcaggaaggatggtgatgtcggctgggtgcagtggctcatgcctgtaattccaatgtgataccctaccttgtgtttaacgtgattgactctcccttagctgagagggccaggcagactctattttggcttcttcgcttgcagtctctcacccaccccccttcctcaaggacttaagctgactcccagcacatccaagaatgcgattactgataagatactgtgacaagctatatccacaattcccaggaattcgtccggttgatagcacccaaagcccccgcgtctatcaccttgtgatagatttaaagcccctgcacctggaactgtttgtttttctgttaccatttatctttttcactttcttgcctgttttgcttctgtaaaattgcttcagctcggctccctcttccccttctaaaccaaggtataaaaagaaacctagccccttctttggggtggagagaattttgagcgctagccgtctctcagtcgccggctaataaaggactcctgaattagtctaa

SEQ ID NO: 2 - DNA, 1476 bp, Homo sapiens
  source 1..1476: mol_type = genomic DNA
cgagactccatctcaaaaacaaaacaaataaacgaacaaaaaaacccacaacgtattattttcttgtttacgaggtttcttgtctctctggctccaccagaagaggagcagggacccttcttgctgttgttcattgctgcatcccccacaccgagagcagagcctggcatgggcagaaagtcctcagtcgatatttggtggccccaagcgaatgaagcatccaagaagggaaagctgggggctccccactgcacttgccacctgagtcacattttcagaagcctctggaaagtcgtgcacagcccaggagtgttgagcaatttcggtttcctctgaggttgaaggacccaggcgtgtcagccctgctccagacaccttgggcatggaggagagtgtcgtacggccctcagtgtttgtggtggatggacagaccgacatcccattcacgaggctgggacgaagccaccggagacagtcgtgcagtgtggcccgggtgggtctgggtctcttgctgttgctgatgggggccgggctggccgtccaaggctggttcctcctgcagctgcactggcgtctaggagagatggtcacccgcctgcctgacggacctgcaggctcctgggagcagctgatacaagagcgaaggtctcacgaggtcaacccagcagcgcatctcacaggggccaactccagcttgaccggcagcggggggccgctgttatgggagactcagctgggcctggccttcctgaggggcctcagctaccacgatggggcccttgtggtcaccaaagctggctactactacatctactccaaggtgcagctgggcggtgtgggctgcccgctgggcctggccagcaccatcacccacggcctctacaagcgcacaccccgctaccccgaggagctggagctgttggtcagccagcagtcaccctgcggacgggccaccagcagctcccgggtctggtgggacagcagcttcctgggtggtgtggtacacctggaggctggggagaaggtggtcgtccgtgtgctggatgaacgcctggttcgactgcgtgatggtacccggtcttacttcggggctttcatggtgtgaaggaaggagcgtggtgcattggacatgggtctgacacgtggagaactcagagggtgcctcaggggaaagaaaactcacgaagcagaggctgggcgtggtggctctcgcctgtaatcccagcactttgggaggccaaggcaggcggatcacctgaggtcaggagttcgagaccagcctggctaacatggcaaaaccccatctctactaaaaatacaaaaattagccggacgtggtggtgcctgcctgtaatccagctactcaggaggctgaggcaggataattttgcttaaacccgggaggcggaggttgcagtgagccgagatcacaccactgcactccaacctgggaaacgcagtgagactgtgcctcaa

SEQ ID NO: 3 - DNA, 4487 bp, Homo sapiens
  source 1..4487: mol_type = genomic DNA
agcgtgcacagcccaggagtgttgagcaatttcggtttcctctgaggttgaaggacccaggcgtgtcagccctgctccagacaccttgggcatggaggagagtgtcgtacggccctcagtgtttgtggtggatggacagaccgacatcccattcacgaggctgggacgaagccaccggagacagtcgtgcagtgtggcccgggtgggtctgggtctcttgctgttgctgatgggggccgggctggccgtccaaggctggttcctcctgcagctgcactggcgtctaggagagatggtcacccgcctgcctgacggacctgcaggctcctgggagcagctgatacaagagcgaaggtctcacgaggtcaacccagcagcgcatctcacaggggccaactccagcttgaccggcagcggggggccgctgttatgggagactcagctgggcctggccttcctgaggggcctcagctaccacgatggggcccttgtggtcaccaaagctggctactactacatctactccaaggtgcagctgggcggtgtgggctgcccgctgggcctggccagcaccatcacccacggcctctacaagcgcacaccccgctaccccgaggagctggagctgttggtcagccagcagtcaccctgcggacgggccaccagcagctcccgggtctggtgggacagcagcttcctgggtggtgtggtacacctggaggctggggagaaggtggtcgtccgtgtgctggatgaacgcctggttcgactgcgtgatggtacccggtcttacttcggggctttcatggtgtgaaggaaggagcgtggtgcattggacatgggtctgacacgtggagaactcagagggtgcctcaggggaaagaaaactcacgaagcagaggctgggcgtggtggctctcgcctgtaatcccagcactttgggaggccaaggcaggcggatcacctgaggtcaggagttcgagaccagcctggctaacatggcaaaaccccatctctactaaaaatacaaaaattagccggacgtggtggtgcctgcctgtaatccagctactcaggaggctgaggcaggataattttgcttaaacccgggaggcggaggttgcagtgagccgagatcacaccactgcactccaacctgggaaacgcagtgagactgtgcctcaaaaaaaagaaaggaagaaaaaagaaaactcaggaaacagatcttgggggacactccagggaacccaaaactcaaaggcggagagctcagtgggcaccaccaaggcgagatgaagccccagcaggcaccttcagaagacccacgtagactgcagaccctgccacggacaatactaaggacaaaaacccagagacttggggtctgtgggcccccaaacatggggtaaagttgatttgcctgatattcaggaagaaggggtgaggggtgggtatttatgcttttgattcagaagaaagtggggcttgggattccagggacttggctgggggtgggaaacttcatccacttccctactctcatcatgagtacggacagggtgggcgggagactgatcatcgggactcatcatgaagagcccagccccaccccacatactcagatcccacccacagactggtggccacacctcagcctggtcacaaagagttacactcagatacatgagcacggcagcgtgctcataactgtttaacaaccagctgtcctgggagggggacagctttgtaatgtttgccaatttccatggtgtaaatgctaccaccatggctgatttcatcactgccaagcatagacatccctaataggacaccacggatctgtccccggcatccggcccagggcctggcacaaagcatgctctagggaaatgcttgctgattgaaaggaaggaagaatgactctacagtcacacctatggcatcccacaaaatctgtcacatggctgcataatctcagccactctttcacaactatagactcatacacgcgaagtgccagattcatgcacaaccacacaatcacatggaagtcacagacggcatcacagacagtcacagcactgtgtgtatgttataacacaagcacacaaaactcagacagcatcccagctacacagccactcccagaggtgtcaccgtcacacttggtaattaatactcattacattagacacagacagaccaagttatagtcagacctggttacacacatacacacacacaatatcaccatgacaaatacacattacacacacacaacatcacaatgacaaacacacattacacacacaacatcacgatgacaaacacacattacacacacaacatcacgatgacaaacacacattacacacacatcacaatgacaaacacaacattacacacacacaacatcacaatgacacacacatcacacacacatcacaatgacaaacacacaacattacacacatatacacacagcctgagggccctccccagcccagactaacacatctcggggtgaggaccagaccttgttcataaccctgggcctcttaaccactgatctttgaaataaatggcaaatagttgtacctggatctgtctagttcttaggggaacaaactgaagaagggtggagaggaattgtcaggcctaaagagccccacagggaaagggaggagtcggatggggggcaaccatcagcaacaagtggtggctcctagaggcagagggatggaggtaatgacccatggaggtcattctacagatgaggaacctggacccagttggctcaagtccatgcaggaaatgtgggggaaaccagagacctcacgtctggatctggcttcctctccaatccacaattcctgaggaagtagaggctacatcccgcaagacgcccttattagacacatccaggacagaatgacaatccgccaagccagctggaagcataaaacacagggagctggtgggttgggtgggggcagataatgatatgcatacaaattagagggtctatgcaaatgagcattgctgcagtgtggctggagggaatccttagttcctaggattctaggatatgggtttcgaccccagaggtgaatgtattgttattattgttttgttgttgttgtgaatgacaagtcaaaatttgtgggttattgttgttatcgccaatagtattcttgtcattgttgcacagtacagagatgaaggaaacagattttgcaatcagatgatcctgggttctgagtccactctgccactcaccagctatatgacctccagcaatttccatcacctctcaatgcttcagtttccccatcggcaagatggttgtggggggagaggaacaacagtacagattcaccatcccaaattcaaaatgctccaaaatctaggccgggcgtggtggctcatacctgtaatcccagcactttgggaggtcaaagtggacggataacctgaggtcaggagctccagaccagcctggccaacatggcgaaaccccatctctactaaaaatacaaaaaattacctgggtgtggtggggggcacctgtaaccccagctactcgggaggctgaggcaggaaccctggaggttgaggttgcagtgagctgagatcacaccactgcactccagcctgggtgacagagcaaggctcccatctcaaaaaacaaaaaaacatgctccaaaatctgaaactctttgagccccagtgtgatgccacaagtgggaaattccacaactcatcacatgtgatagattgcagtggaaatgcaggcacacaccacgaagtttactcagcatcctcaaaggaaatccccgtcagtagctatatatcattttctcacatgccagataggtatctctcatcttttactgttaggtacttctgtgttgaataggtggaggaaaatgattgctggttagtagtatataaattcagagtcaggaaggatggtgatgtcggctgggtgcagtggctcatgcctgtaattccaatgtgataccctaccttgtgtttaacgtgattgactctcccttagctgagagggccaggcagactctattttggcttcttcgcttgcagtctctcacccaccccccttcctcaaggacttaagctgactcccagcacatccaagaatgcgattactgataagatactgtgacaagctatatccacaattcccaggaattcgtccggttgatagcacccaaagcccccgcgtctatcaccttgtgatagatttaaagcccctgcacctggaactgtttgtttttctgttaccatttatctttttcactttcttgcctgttttgcttctgtaaaattgcttcagctcggctccctcttccccttctaaaccaaggtataaaaagaaacctagccccttctttggggtggagagaattttgagcgctagccgtctctcagtcgccggctaataaaggactcctgaattagtctaa

SEQ ID NO: 4 - DNA, 6396 bp, Homo sapiens
  source 1..6396: mol_type = genomic DNA
actcgctctataggtagcaagacccgttgtcctttaggaatacggaggtttacatcttcgttctgagggtgggggaaaaatcagttgtcactttaaaagagttcgcgcttgctaaggtactaaggcagaagccgcaccgaagcgtcgcgataactgcaaccacccgcaacttctcgcgatgtttggccccgctaaaggtcgccattttggagtccacccggcgcctggtttccccggcggcgtctcccaacaggctgccgggaccaaagctggccccgcgggtgcctggcctgtgggcagccggaccgacacgatgtggcggctccgctgcaaggccaaggacggcacccatgttttgcaggggctgtccagccggacccgggtgcgggaactccagggccaaattgccgccatcaccgggatcgcccccggcggtcagcgaatcctcgtcggataccctcccgagtgcctggatctcagcaatggggataccattctggaagacttgcccatccaatctggtgacatgctgatcattgaagaagaccaaaccaggcccagaagttcacctgcatttactaaacgtggtgcttctagttacgtcagggaaactttgcctgtgcttaccagaaccgtggtcccagcagacaactcttgcctctttactagtgtgtactatgtcgtcgaaggaggagtcttgaatccagcttgtgcccctgagatgagacgcctcatagcacaaattgtagcaagcgatccagacttctatagtgaggcaatactgggaaaaacaaatcaagagtactgtgactggatcaaaagggatgacacttggggaggagcaatagagatatcgattttgtccaagttttaccaatgtgaaatatgtgtagtggatacacagacagtaagaattgatcgttttggggaagatgcaggatataccaaaagggttctgcttatttatgatggcatccactatgatccacttcagcgtaacttccctgatccagatacacctcctctgaccattttctcctctaatgatgatattgttcttgtacaagcactggaattagcagatgaagctagaagaaggagacagtttactgatgtcaaccgcttcaccctgagatgcatggtatgtcagaaaggattaactggacaagcagaagcaagggaacatgccaaggagacaggccataccaactttggagaagtgtgacctatgcatgaatgagggttgaagcctactacctcacacatccagaaggctctgggttttccaataagctatggtaaccctaaagaacaaaggatacaatgcttgaaccatccttttaacttaaaaccactaagacactgaaattccttgttaagattaaaattagtgtgcaagtttacagatgtgtgtctacagtggtaaactgtacatacatgcctctttctgctggagtgacagaataggtgatccttgccacctactgacactgacctgaaggttgagattgagtattataaactagcacccagcagctttaacttgtagaagaaagcatcacattttgggtaatgtggaaggcctcctgtgagtccactgggcatacgattgagattgagtattataaactagcacccagcagctttaacttgtagaagaaagcatcacattttgggtaatgtggaaggcctcctgtgagtccactggacatttaccacagtgtctccagtaactgagtctttttaaaaactctgaatgagttaagtttctaaattatgaattgattcatcaaatgaagatactcagaattgtccaaactgattttatattgcaatttggtagacattataaatgtgtgcttaaccactgataagtacatcacaagcaatttttacagggatgagtctcatccttgagaatgttatcacaaaacaggaactgattgtgccctgtttaagatctctagcatataaaacgtagaatgtatgagggaataggtgcctgagcagcttcctgaagctttaaaagaccgttggcctcgtgttttaatgcaattcatgtattggtctttgtcacattggataacattttaaagttaagcagggtacttttttaattgaaattccttgaaattcgagtcctcagttttttcttcatttgcgtaaagtttatcggggggaatttaattttctcagctttttgttaagagcacttcctccaaaaaatttttttcaagtaataatgctctgctttgggttggtttttgtaagattttttgcacacctaaagagtgtttgcttttgtgctagccttatccctccactaaagttattttaaataatttcacatttctgcaaattagcactttgcttatctgcaatcttttactttgatttttgaagttttaaagcaattggagtaatactgttgaatgaactagtttcacttccaaaatagaaaaaattgtaaatccttgccttatgcagctttctcagaattctgcttcttcctagtactagatgtgtagccatttgcttagtggactaatccgcaaggcacaccctctaaaacttagcttcactacaagatcttccagataaaagttttctacctcttttcttaattattctgatcagggatgctaaattataatttgttatgtattatctcacataatgtgaagaggcttaatgtgaagttttgttattttggtctcttttttattaagtatctcacttagaaattcagtggtatactttaaagcacttggatctttttcagcatatctgcctagcaaatgttttaaaattgacatttatttttagcactttcacttggtgaaggtggccatataaaattaaggaacatttgaacaatataagagaaaagaacttttaaggaacaattcacaaagtttgtttgaaattgtcagatgacatttcttgagtaccttttgtgtgcatagttattttagacaatataagctgttatggtcagcataacttaaaagtgtttagttttctattttactgagccttaaaaatagcactgatgagcttatgatacttaatgtttggcaatcataatgtgttcaaattaatgggattgaaaatctctccacacctgactctcatctgatctggatggttttggttttgtatcttttttacttctcccagaaaatactaaatttaaaactgtaaattaagaatataccactagataacaattatcaaattgagctttatgcatcattactcagaaagcttgccttcctttctttgctacttcaggacacagagttgacatttgcttactacagctttagatctagaagtttattcgtgcaacaaatatttattgagtaatttatactgtgccaggcatgttttgatatgtttctgtcatatgttttgatatgttccaacataagtttctgtcactttatattcagtatatattttctacagtgggtaaatttaacaaatggaaaggaatagaacactgatattttacagaattaaaccccttcattgtaagggctttgtttacatattaagtgtcaagtatttattcaggggatcttatttcattgtattttatctgttatctaggttgtccatttaccggttggacactgatactctgtcaaattcctttcaaaaatgactctttagtctgctgaaatttagcactagtactttagtgttctgatcctggaaaattcaaggtgaagctttatttgtggaccatctgatttaattattgaggattaaaaacctaaacctttgctcattctaaactcaagcttttaagcctcacagaatttacaggggtttgctttttgtttgtttgttttttcattttttactgtgcttattaaactcttggaattagttattaaagggagtaaattctcatcttgggaattttgaaaatctatggacttacaactttcaggaggattaaatgtcttaagttttgtactagagcagaatgaaatctttcctattcattgagtttttgcctgccatagaggaatttttttaaaaattaaaatgacagtttatattagtggcaaagtgaataaagacctcactttcccaccccacccttcttcctttctcttacttttctttggattaaaggtcaggtgtagtactatgaagattcactcctgaataaagtgatttcagaagctaaaatttaacatacctggaaattttgtgatgtgttagccaagtgaagacattagtgtgttccatcttttgctaatggttcatggttgatttcttcattgtttcccatgaaattagcatagtcaagtggtacccttgacgcttgactgctggtcagtttgaccctgtttttaacaactaatgtagtcatgccgcttgattattccatgaagtcccagcaaaataataatgaggaattaactaacattatgttatctatctaatttgtctgtgtccctaaatgcccatgcctaacttgcttctctagtttattccttctgtggagggattaaaacgtgggtgttgcaagttgccctaagctaaacatagttttcttacatctttttgggaaaaaaaatggaatgggaagtatgcaagattaagcaagagtgatttttttttttttttgacaaatcaggtggccttcctaaacatactaagaattatgttctttcatgtgtggagacacatttgtttgcagcactttaaaaaatatatatggaataaaagtttacatgttggccctctagggatctaattaaggacattaaagtacaattcttgagctactaaccatcagctcttcttaatcaaagattgccatcagtgtagagtgtatctattggcacaacattctggtgttttgataacagtagaactcaatttcagtaactattaggagcatggtctgtgccctagcattaaaaatgttacttattattatgtgaatatcttgtattattatacaatgcagtattcaaatttgtccttgtagtgcagagatgactgataatttctaaaagattcgatccttaaaacttgtttccaagcagacttataaggaagctgatttttgagtcagaggccttaaacgtgtcatatacaagtggcatcattttaagtccaaagtgaaacacttgatttgaataagctagtttataaactaaagctgttttcttatgttacagtatttcagcacatttcattccacataaaaagaatattaagtgtccctggttgtgggagagtgtttatttttctcaaaattatctagcattttgcttacagtgctttgaatgtttgacttaaaattattattgatgttgaattgtagggtgctgatttaggtcttgattcatacacatttaaaggaggttggtaaccccctcatggtagagtgaagggagaaaagggccaagaagacaaagtaccactgataaagaagagattgtcaaatagatgcattcctagtcatgaattacccttttccaaacatttttaaagcaatgcctttgtgtcaactcaacccttcttccccatttcttgtcatagaatgtagcatggccataggtgaaaaagcttatcattaaagtatgaaaccatgaattataagcattttgccatgatgcccttttatacatatgtttttaaaagtactaaccaacatataggagtttaggaatggtgaagatataatttgattaagttgtaggtaaacagaaaggatcatcttaggctcagaatttctaatatgattacatgagtctactttataaactggtataggctatgtaattagcccgtaagttacttaaaggaccaggggacctaatttttgtcagttttccagtcacattggtgccattcaggactccagctgtttacaggaaatatgtacttagcagaatagtatttttccttgaaaaaaatttgaattcagcctaaatacagaatgaatatgaatagtttgtgaaaagggttagagaacaacaatattcctatagtttctgtattaatgcagtagagacagaggttcctaacgcaaaaagaaaaccacaagtaaagaccgtcaaattagagctttagaatatgacttgaaaaagtagggatgggcaaaacagcataagaaaatattttttcttaatgcagatggacagtgttttcttgttttaaaaatgttttgcctatttgccagcattttttgaagtaatacactgctgctacctggaagatgtctaacttcattttctacaactcttatgtgattttgccattgtcattaagatgcattgattttatttatgaggtgtatgactttaaatatctaaatgctgtattaagtgacttgtttcaaaggaataaatgaagtgaaaacgt

SEQ ID NO: 5 - DNA, 6291 bp, Homo sapiens
  source 1..6291: mol_type = genomic DNA
agactattcggtaggcgtcttgagagcgggtgtgccgggtgacgagaaaatgctgcaaagattaacgctctcattcctgaatcccagcagaacctcattagatccataaatgggaacgctgtatcatccgttgcagtcgtcttgaagaaccaaggaggaaaattgcaccagcaaaaaaaaattgagtcatgaaagatgtgaaaagatggaaacattacatataatttattcagaagcaaagtcttttacagtggaggggctgtccagccggacccgggtgcgggaactccagggccaaattgccgccatcaccgggatcgcccccggcggtcagcgaatcctcgtcggataccctcccgagtgcctggatctcagcaatggggataccattctggaagacttgcccatccaatctggtgacatgctgatcattgaagaagaccaaaccaggcccagaagttcacctgcatttactaaacgtggtgcttctagttacgtcagggaaactttgcctgtgcttaccagaaccgtggtcccagcagacaactcttgcctctttactagtgtgtactatgtcgtcgaaggaggagtcttgaatccagcttgtgcccctgagatgagacgcctcatagcacaaattgtagcaagcgatccagacttctatagtgaggcaatactgggaaaaacaaatcaagagtactgtgactggatcaaaagggatgacacttggggaggagcaatagagatatcgattttgtccaagttttaccaatgtgaaatatgtgtagtggatacacagacagtaagaattgatcgttttggggaagatgcaggatataccaaaagggttctgcttatttatgatggcatccactatgatccacttcagcgtaacttccctgatccagatacacctcctctgaccattttctcctctaatgatgatattgttcttgtacaagcactggaattagcagatgaagctagaagaaggagacagtttactgatgtcaaccgcttcaccctgagatgcatggtatgtcagaaaggattaactggacaagcagaagcaagggaacatgccaaggagacaggccataccaactttggagaagtgtgacctatgcatgaatgagggttgaagcctactacctcacacatccagaaggctctgggttttccaataagctatggtaaccctaaagaacaaaggatacaatgcttgaaccatccttttaacttaaaaccactaagacactgaaattccttgttaagattaaaattagtgtgcaagtttacagatgtgtgtctacagtggtaaactgtacatacatgcctctttctgctggagtgacagaataggtgatccttgccacctactgacactgacctgaaggttgagattgagtattataaactagcacccagcagctttaacttgtagaagaaagcatcacattttgggtaatgtggaaggcctcctgtgagtccactgggcatacgattgagattgagtattataaactagcacccagcagctttaacttgtagaagaaagcatcacattttgggtaatgtggaaggcctcctgtgagtccactggacatttaccacagtgtctccagtaactgagtctttttaaaaactctgaatgagttaagtttctaaattatgaattgattcatcaaatgaagatactcagaattgtccaaactgattttatattgcaatttggtagacattataaatgtgtgcttaaccactgataagtacatcacaagcaatttttacagggatgagtctcatccttgagaatgttatcacaaaacaggaactgattgtgccctgtttaagatctctagcatataaaacgtagaatgtatgagggaataggtgcctgagcagcttcctgaagctttaaaagaccgttggcctcgtgttttaatgcaattcatgtattggtctttgtcacattggataacattttaaagttaagcagggtacttttttaattgaaattccttgaaattcgagtcctcagttttttcttcatttgcgtaaagtttatcggggggaatttaattttctcagctttttgttaagagcacttcctccaaaaaatttttttcaagtaataatgctctgctttgggttggtttttgtaagattttttgcacacctaaagagtgtttgcttttgtgctagccttatccctccactaaagttattttaaataatttcacatttctgcaaattagcactttgcttatctgcaatcttttactttgatttttgaagttttaaagcaattggagtaatactgttgaatgaactagtttcacttccaaaatagaaaaaattgtaaatccttgccttatgcagctttctcagaattctgcttcttcctagtactagatgtgtagccatttgcttagtggactaatccgcaaggcacaccctctaaaacttagcttcactacaagatcttccagataaaagttttctacctcttttcttaattattctgatcagggatgctaaattataatttgttatgtattatctcacataatgtgaagaggcttaatgtgaagttttgttattttggtctcttttttattaagtatctcacttagaaattcagtggtatactttaaagcacttggatctttttcagcatatctgcctagcaaatgttttaaaattgacatttatttttagcactttcacttggtgaaggtggccatataaaattaaggaacatttgaacaatataagagaaaagaacttttaaggaacaattcacaaagtttgtttgaaattgtcagatgacatttcttgagtaccttttgtgtgcatagttattttagacaatataagctgttatggtcagcataacttaaaagtgtttagttttctattttactgagccttaaaaatagcactgatgagcttatgatacttaatgtttggcaatcataatgtgttcaaattaatgggattgaaaatctctccacacctgactctcatctgatctggatggttttggttttgtatcttttttacttctcccagaaaatactaaatttaaaactgtaaattaagaatataccactagataacaattatcaaattgagctttatgcatcattactcagaaagcttgccttcctttctttgctacttcaggacacagagttgacatttgcttactacagctttagatctagaagtttattcgtgcaacaaatatttattgagtaatttatactgtgccaggcatgttttgatatgtttctgtcatatgttttgatatgttccaacataagtttctgtcactttatattcagtatatattttctacagtgggtaaatttaacaaatggaaaggaatagaacactgatattttacagaattaaaccccttcattgtaagggctttgtttacatattaagtgtcaagtatttattcaggggatcttatttcattgtattttatctgttatctaggttgtccatttaccggttggacactgatactctgtcaaattcctttcaaaaatgactctttagtctgctgaaatttagcactagtactttagtgttctgatcctggaaaattcaaggtgaagctttatttgtggaccatctgatttaattattgaggattaaaaacctaaacctttgctcattctaaactcaagcttttaagcctcacagaatttacaggggtttgctttttgtttgtttgttttttcattttttactgtgcttattaaactcttggaattagttattaaagggagtaaattctcatcttgggaattttgaaaatctatggacttacaactttcaggaggattaaatgtcttaagttttgtactagagcagaatgaaatctttcctattcattgagtttttgcctgccatagaggaatttttttaaaaattaaaatgacagtttatattagtggcaaagtgaataaagacctcactttcccaccccacccttcttcctttctcttacttttctttggattaaaggtcaggtgtagtactatgaagattcactcctgaataaagtgatttcagaagctaaaatttaacatacctggaaattttgtgatgtgttagccaagtgaagacattagtgtgttccatcttttgctaatggttcatggttgatttcttcattgtttcccatgaaattagcatagtcaagtggtacccttgacgcttgactgctggtcagtttgaccctgtttttaacaactaatgtagtcatgccgcttgattattccatgaagtcccagcaaaataataatgaggaattaactaacattatgttatctatctaatttgtctgtgtccctaaatgcccatgcctaacttgcttctctagtttattccttctgtggagggattaaaacgtgggtgttgcaagttgccctaagctaaacatagttttcttacatctttttgggaaaaaaaatggaatgggaagtatgcaagattaagcaagagtgatttttttttttttttgacaaatcaggtggccttcctaaacatactaagaattatgttctttcatgtgtggagacacatttgtttgcagcactttaaaaaatatatatggaataaaagtttacatgttggccctctagggatctaattaaggacattaaagtacaattcttgagctactaaccatcagctcttcttaatcaaagattgccatcagtgtagagtgtatctattggcacaacattctggtgttttgataacagtagaactcaatttcagtaactattaggagcatggtctgtgccctagcattaaaaatgttacttattattatgtgaatatcttgtattattatacaatgcagtattcaaatttgtccttgtagtgcagagatgactgataatttctaaaagattcgatccttaaaacttgtttccaagcagacttataaggaagctgatttttgagtcagaggccttaaacgtgtcatatacaagtggcatcattttaagtccaaagtgaaacacttgatttgaataagctagtttataaactaaagctgttttcttatgttacagtatttcagcacatttcattccacataaaaagaatattaagtgtccctggttgtgggagagtgtttatttttctcaaaattatctagcattttgcttacagtgctttgaatgtttgacttaaaattattattgatgttgaattgtagggtgctgatttaggtcttgattcatacacatttaaaggaggttggtaaccccctcatggtagagtgaagggagaaaagggccaagaagacaaagtaccactgataaagaagagattgtcaaatagatgcattcctagtcatgaattacccttttccaaacatttttaaagcaatgcctttgtgtcaactcaacccttcttccccatttcttgtcatagaatgtagcatggccataggtgaaaaagcttatcattaaagtatgaaaccatgaattataagcattttgccatgatgcccttttatacatatgtttttaaaagtactaaccaacatataggagtttaggaatggtgaagatataatttgattaagttgtaggtaaacagaaaggatcatcttaggctcagaatttctaatatgattacatgagtctactttataaactggtataggctatgtaattagcccgtaagttacttaaaggaccaggggacctaatttttgtcagttttccagtcacattggtgccattcaggactccagctgtttacaggaaatatgtacttagcagaatagtatttttccttgaaaaaaatttgaattcagcctaaatacagaatgaatatgaatagtttgtgaaaagggttagagaacaacaatattcctatagtttctgtattaatgcagtagagacagaggttcctaacgcaaaaagaaaaccacaagtaaagaccgtcaaattagagctttagaatatgacttgaaaaagtagggatgggcaaaacagcataagaaaatattttttcttaatgcagatggacagtgttttcttgttttaaaaatgttttgcctatttgccagcattttttgaagtaatacactgctgctacctggaagatgtctaacttcattttctacaactcttatgtgattttgccattgtcattaagatgcattgattttatttatgaggtgtatgactttaaatatctaaatgctgtattaagtgacttgtttcaaaggaataaatgaagtgaaaacgt

SEQ ID NO: 6 - DNA, 1478 bp, Homo sapiens
  source 1..1478: mol_type = genomic DNA
ccttttgctgattttgcctcacagaattgagagtttgttcttacacacaagtttaatgccaccttcctctgtctgccatggaccaacaagcaatatatgctgagttaaacttacccacagactcaggcccagaaagttcttcaccttcatctcttcctcgggatgtctgtcagggttcaccttggcatcaatttgccctgaaacttagctgtgctgggattattctccttgtcttggttgttactgggttgagtgtttcagtgacatccttaatacagaaatcatcaatagaaaaatgcagtgtggacattcaacagagcaggaataaaacaacagagagaccgggtctcttaaactgcccaatatattggcagcaactccgagagaaatgcttgttattttctcacactgtcaacccttggaataacagtctagctgattgttccaccaaagaatccagcctgctgcttattcgagataaggatgaattgatacacacacagaacctgatacgtgacaaagcaattctgttttggattggattaaatttttcattatcagaaaagaactggaagtggataaacggctcttttttaaattctaatgacttagaaattagaggtgatgctaaagaaaacagctgtatttccatctcacagacatctgtgtattctgagtactgtagtacagaaatcagatggatctgccaaaaagaactaacacctgtgagaaataaagtgtatcctgactcttgactatgaatcccatctcaatttatttgcttcccattactgatctctgtacttgtagctgcacatactattggtactacctaatagtgccacatttagtggcacaaagtgaacaattctgagaattgacaactgttatgaatcttacagaagttcatgtttatcatattcattctattaaatgaggaaacagagacatagagaaaaacgtgcatcgttttaaagaaacagtgatattctatggtgaaggagtgaaggatgtccccgaatatgccagattggtatatgattgttttgtgtttaaaacagtggagaaattgtagattcagaaagggagagctgacctgtctcttcccgcacgcggcaagccgtgaagattcctctgggagggctatccgagtcatacaagggcaagaaaatagctcttatcgccagagacctggaattggatgctgcaatgaacctgaataaagatacttaataaacacctatctttcacctattttacagccccccgcaaccaatatatctcctagtgactcctctagaaaatttattgcccctagccagcttttcttcatcctgtcatttcttttcaaatttatcattcttggtctaaaaagcataaaagcatcttgcttaggccacttctatggatttcactctcttgcgagttcctcatgtacatgcaaaacgaataaaatgtgtatacttttattttgttca

SEQ ID NO: 7 - DNA, 841 bp, Homo sapiens
  source 1..841: mol_type = genomic DNA
aagaaagcagaagctctcttcccattatgacttcggaaatcacttatgctgaagtgaggttcaaaaatgaattcaagtcctcaggcatcaacacagcctcttctgcagagacagcctggagctgttgcccaaagaattggaagtcatttagttccaactgctactttatttctactgaatcagcatcttggcaagacagtgagaaggactgtgctagaatggaggctcacctgctggtgataaacactcaagaagagcaggatttcatcttccagaatctgcaagaagaatctgcttattttgtggggctctcagatccagaaggtcagcgacattggcaatgggttgatcagacaccatacaatgaaagttccacattctggcatccacgtgagcccagtgatcccaatgagcgctgcgttgtgctaaattttcgtaaatcacccaaaagatggggctggaatgatgttaattgtcttggtcctcaaaggtcagtttgtgagatgatgaagatccacttatgaactgaacattctccatgaacaggtggttggattggtatctgtcattgtagggatagataataagctcttcttattcatgtgtaagggaggtccatagaatttaggtggtctgtcaactattctacttatgagagaattggtctgtacattgactgattcactttttcataaagtgagcatttattgagcattttttcatgtgccagagcctgtactggaggcccccattgtgcacacatggagagaacatgagtctctcttaatttttatctggttgctaaagaattatttaccaataaaattatatgatgtggtgt

SEQ ID NO: 8 - DNA, 615 bp, Homo sapiens
  source 1..615: mol_type = genomic DNA
atgacttcggaaatcacttatgctgaagtgaggttcaaaaatgaattcaagtcctcaggcatcaacacagcctcttctgcagcttccaaggagaggactgcccctcacaaaagtaataccggattccccaagctgctttgtgcctcactgttgatatttttcctgctattggcaatctcattctttattgcttttgtcaagacagcctggagctgttgcccaaagaattggaagtcatttagttccaactgctactttatttctactgaatcagcatcttggcaagacagtgagaaggactgtgctagaatggaggctcacctgctggtgataaacactcaagaagagcaggatttcatcttccagaatctgcaagaagaatctgcttattttgtggggctctcagatccagaaggtcagcgacattggcaatgggttgatcagacaccatacaatgaaagttccacattctggcatccacgtgagcccagtgatcccaatgagcgctgcgttgtgctaaattttcgtaaatcacccaaaagatggggctggaatgatgttaattgtcttggtcctcaaaggtcagtttgtgagatgatgaagatccacttatga

SEQ ID NO: 9 - DNA, 597 bp, Homo sapiens
  source 1..597: mol_type = genomic DNA
atgacttcggaaatcacttatgctgaagtgaggttcaaaaatgaattcaagtcctcaggcatcaacacagcctcttctgcagttttctttcaaaaatattctcagcttcttgaaaaaaagactacaaaagagctggttcatacaacattggagtgtgtgaaaaaaaatatgcccgtggaagagacagcctggagctgttgcccaaagaattggaagtcatttagttccaactgctactttatttctactgaatcagcatcttggcaagacagtgagaaggactgtgctagaatggaggctcacctgctggtgataaacactcaagaagagcaggatttcatcttccagaatctgcaagaagaatctgcttattttgtggggctctcagatccagaaggtcagcgacattggcaatgggttgatcagacaccatacaatgaaagttccacattctggcatccacgtgagcccagtgatcccaatgagcgctgcgttgtgctaaattttcgtaaatcacccaaaagatggggctggaatgatgttaattgtcttggtcctcaaaggtcagtttgtgagatgatgaagatccacttatga

SEQ ID NO: 10 - DNA, 1296 bp, Homo sapiens
  source 1..1296: mol_type = genomic DNA
gcatttgtttcaaggctgtgattctcactatactggtcctgaggaaagggcttctgtgaactgcggtttttagtttttattgtggttcttagttctcatgagacccctcttgaggatatgtgcctatctggtgcctctgctctccactagttgagtgaaaggaaggaggtaatttaccaccatgtttggttcctgtttataagatgttttaagaaagatctgaaacagattttctgaagaaagcagaagctctcttcccattatgacttcggaaatcacttatgctgaagtgaggttcaaaaatgaattcaagtcctcaggcatcaacacagcctcttctgcagcttccaaggagaggactgcccctcacaaaagtaataccggattccccaagctgctttgtgcctcactgttgatatttttcctgctattggcaatctcattctttattgcttttgtcattttctttcaaaaatattctcagcttcttgaaaaaaagactacaaaagagctggttcatacaacattggagtgtgtgaaaaaaaatatgcccgtggaagagacagcctggagctgttgcccaaagaattggaagtcatttagttccaactgctactttatttctactgaatcagcatcttggcaagacagtgagaaggactgtgctagaatggaggctcacctgctggtgataaacactcaagaagagcaggatttcatcttccagaatctgcaagaagaatctgcttattttgtggggctctcagatccagaaggtcagcgacattggcaatgggttgatcagacaccatacaatgaaagttccacattctggcatccacgtgagcccagtgatcccaatgagcgctgcgttgtgctaaattttcgtaaatcacccaaaagatggggctggaatgatgttaattgtcttggtcctcaaaggtcagtttgtgagatgatgaagatccacttatgaactgaacattctccatgaacaggtggttggattggtatctgtcattgtagggatagataataagctcttcttattcatgtgtaagggaggtccatagaatttaggtggtctgtcaactattctacttatgagagaattggtctgtacattgactgattcactttttcataaagtgagcatttattgagcattttttcatgtgccagagcctgtactggaggcccccattgtgcacacatggagagaacatgagtctctcttaatttttatctggttgctaaagaattatttaccaataaaattatatgatgtggtgtctc

SEQ ID NO: 11 - DNA, 349 bp, Homo sapiens
  source 1..349: mol_type = genomic DNA
ttcaaaaatgaattcaagtcctcaggcatcaacacagcctcttctgcagcttccaaggagaggactgcccctcacaaaagtaataccggattccccaagctgctttgtgcctcactgttgatatttttcctgctattggcaatctcattctttattgcttttgtcagatttcatcttccagaatctgcaagaagaatctgcttattttgtggggctctcagatccagaaggtcagcgacattggcaatgggttgatcagacaccatacaatgaaagttccacattctggcatccacgtgagcccagtgatcccaatgagcgctgcgttgtgctaaattttcgtaaatca

SEQ ID NO: 12 - DNA, 5134 bp, Homo sapiens
  source 1..5134: mol_type = genomic DNA
atttggagcatttccttccctgacagccggacctgggactgggctggggccctggcggatggagacatgctgcccctgctgctgctgcccctgctgtggggggggtccctgcaggagaagccagtgtacgagctgcaagtgcagaagtcggtgacggtgcaggagggcctgtgcgtccttgtgccctgctccttctcttacccctggagatcctggtattcctctcccccactctacgtctactggttccgggacggggagatcccatactacgctgaggttgtggccacaaacaacccagacagaagagtgaagccagagacccagggccgattccgcctccttggggatgtccagaagaagaactgctccctgagcatcggagatgccagaatggaggacacgggaagctatttcttccgcgtggagagaggaagggatgtaaaatatagctaccaacagaataagctgaacttggaggtgacagccctgatagagaaacccgacatccactttctggagcctctggagtccggccgccccacaaggctgagctgcagccttccaggatcctgtgaagcgggaccacctctcacattctcctggacggggaatgccctcagccccctggaccccgagaccacccgctcctcggagctcaccctcacccccaggcccgaggaccatggcaccaacctcacctgtcaggtgaaacgccaaggagctcaggtgaccacggagagaactgtccagctcaatgtctcctatgctccacagaacctcgccatcagcatcttcttcagaaatggcacaggcacagccctgcggatcctgagcaatggcatgtcggtgcccatccaggagggccagtccctgttcctcgcctgcacagttgacagcaacccccctgcctcactgagctggttccgggagggaaaagccctcaatccttcccagacctcaatgtctgggaccctggagctgcctaacataggagctagagagggaggggaattcacctgccgggttcagcatccgctgggctcccagcacctgtccttcatcctttctgtgcagagaagctcctcttcctgcatatgtgtaactgagaaacagcagggctcctggcccctcgtcctcaccctgatcaggggggctctcatgggggctggcttcctcctcacctatggcctcacctggatctactataccaggtgtggaggcccccagcagagcagggctgagaggcctggctgagcccctcccgctcaagacagaactgaggtgtggacacttagccctgtgggacacatgcaggacatcactgtcagcttctttctggaagctcacatcccactgactacccctcttttccttcctgccccataccccttctacttattcccctctgcttgtgagtcttgccccaccacacctgcatccccatctgcaccccatcccctctccacctgcccttctcttccctctccatccaccatctccagccctgtgaagggaatgtactttcggtcttatacccccattacccattacccaaaagttaccttttttttttttttttttttttgagacagagtctcactctgttgcacaggctggagttcagtggcacaatctccgttcactgcaacctccacctctggggttcaagcaattctcctgcctcagcctccctagtagctgggattacaggtgcctgccaccacatccagttaattttttttttttgtatgttagtagagatggggttttaccatgttggccaggtctcgaactcctgacctcaagcaatccactgcattggcctcccaaagtgctggcattacaggtatgagccaccgtgcctggctgccaaaagttaccttcttaacacttgaatttctggtctcctcagcttccctatccatataggcacagagaggcagcatttgttttccagttaaaactctacctcattgtgattattatccaatacaattgttacaaaataagtaaaacttttatgaaacaatacaacataactgattttactctttaatgcctctgtgagagtttgtagacaaaaattatgtcttttttttttttctttgagacagagtttctatcttgttgcccaggctggagtgcaatggcaaaatctcagctcactgcaacttctgcctcccaggttcaagtgattctccttctgtccatatacaagaaggcaatacctgtattgtcaggttctgtgcatcgtataactggaaccaaacatatttgctttagggtctgctttcatttcttcagtgtggttttcccagtttatccacgttgttacacgtatcaatagctcattctcagttttggtggggttttttttgcttttaatatcgtacagtcagccttctgtatccactggttctgcattttccctttaatcacttttgctgcaccacaaaagttttgttatgttgtatttttatattagttcaaaatatttccttctttcccctgagatttcctttgaattcacggattgcttagaagtgtgttgtttaatttctaagtgattgcagattttactggttttttatttttaaacaaattgttactactttctttttaagttccattttaataaatacacatgcttgatatgattttttttaacttttaagttcagggggcacaagtgcaggtttgttacataggtaaagtgtcatgggagtttgttgtacagattattgcatcacccagatattaagcctagtacccattagttattttcctcatcctctccctcctcccaccttccaccctttgaaaggccccagtgtgtgttgctcacctctatgtatccatgtgttctcatcatttagctcccacttacaagtgagaacatgtggtatttggttttctcttcttgtgatagtttgctgaggataatggtctccagctccactcatgtccctgcaaaggacataatctcattcttttttatggctgcttagtattccatggtgtatatgtaccacattttctctatccagtctaccactgataggcagttaggttgattccatgtcattgctattgtgaatagtgctgcagtgaatgtatgcatgcatgtgtctttgtaatagaatgatttatattcctttgggtatatgcctaggaatgggattgctgagtcgaatggtatttctatgtttaggtctttgaggaatcgccacactgtcttccacaatggctgaactaactttcactttcaccaaccgtgagagtcttttatattggttaagtttgcttgatgacactggtctatcttggtgaatgctccatgtgtgcttagaaagaatgtgtattgccctgttatgggacgaatattaaatggcaattagacatagttgtccaatggtgttcagttttatagctggtaacttttttgtctaccagctcagtctattactgagagaggaatgttgaagtctctgatcctaatgttggatttgtcagtttctcctctcagtttcatcagtttttgctgcatgtatttttaaactctgtcgttaggtgcatacatattaagaattctcatgtcttcttaaagaatcaacttaaaaaaaatttttttttgagacagagtttcgctctttttgcccaggctggagtgcaatggcgcgatcttggctcactgcaacctccgcctcccaggtacaagtgattctcctgcctcagcctcccaaatagcttggattacaggcacgcaccatcacgcctggctagttttttttgtatttagtagagacaaggtttcaccatgtaagtcaggctggtcctgaactcctgacttcaggtgatccacccgcctcagcctccaaagtgctgggattataggcgtgagccaccgcagttggctgaatcaactgttttacattatgtaacatcactttttgttcctgtgattttctttgctcttaagtgtactttgtctgctattaacatagccattccagttttcttttgactagtatttgcatagtatgcattttcacatcctttaagtcctagcctcacctcattatatttgaaatggaaagcatttatactcagaagctggagttccttttccctagctcttccctttccagaattgttacctgttgtttcagtgttcctagttgccctgggcttcatcccttgtttctcagtccagaaagatggaaggagttgtattagaattttagcagccactttctgcactgtagctctgacctaccattggaataaagctatttattccttgttggtgcctttccccaaatattgactcccgttccagaatctattttcttttatcccatttcccaagtagttttttttccccattcaaagcttataacttgtaaggattttttgtttgtttgttttgttgtgttgtggtgagttcactctgctaggagcttactccttcataataaaagcacgactccttctctttcgttttgaaggataattttccaaaatgtagaattctagctttgcatttttcttttaaccttttggagatgtcattccactttggagggcgggtgagtttctcatgacaattcagtcatcattttcttattgtggttccatttaaggcaatatctgtttatgtcttgctgcttttataatttcttcattctttttcatgaatttaacttttataaacttcaggtgtttttcttttaatttccctaagtgcatgtagcaaagagagtgcaatatttgctttttttctatatgctttaactcttgatatactttatttatgctataatagaaatgtgtgtcttcccaaaatttatatgttgaaatcttaaacctcaaggtgatggtattaaaaggttggggctttttggaaagtgattaacccataatggtgccatccttcatgaatgggattagtgttctcataaaagaaacagaaggaagtgtgttttcctcttctgccatgtgaggataccacgaaaagatactatctgggaagcaaataattctctccagacactgaatccgctggcaccttgatcttggacttcccgacctccagaattatgagaaataaatttctgttgtttataaatca

SEQ ID NO: 13 - DNA, 596 bp, Homo sapiens
  source 1..596: mol_type = genomic DNA
atccctcttgtcacctctgaagctggtgctgtatctttctatcccagatgctccacagaacctcgccatcagcatcttcttcagaaatggcacaggcacagccctgcggatcctgagcaatggcatgtcggtgcccatccaggagggccagtccctgttcctcgcctgcacagttgacagcaacccccctgcctcactgagctggttccgggagggaaaagccctcaatccttcccagacctcaatgtctgggaccctggagctgcctaacataggagctagagagggaggggaattcacctgccgggttcagcatccgctgggctcccagcacctgtccttcatcctttctgtgcagagaagctcctcttcctgcatatgtgtaactgagaaacagcagggctcctggcccctcgtcctcaccctgatcaggggggctctcatgggggctggcttcctcctcacctatggcctcacctggatctactataccaggtgtggaggcccccagcagagcagggctgagaggcctggctgagcccctcccgctcaagacagaactgagtagagatggggttttaccatgttggccaggt

SEQ ID NO: 14 - DNA, 50 bp, synthetic construct
  source 1..50: mol_type = other DNA
gggtctgacacgtggagaactcagagggtgcctcaggggaaagaaaactc

SEQ ID NO: 15 - DNA, 50 bp, synthetic construct
  source 1..50: mol_type = other DNA
cagttttccagtcacattggtgccattcaggactccagctgtttacagga

SEQ ID NO: 16 - DNA, 50 bp, synthetic construct
  source 1..50: mol_type = other DNA
cagtctagctgattgttccaccaaagaatccagcctgctgcttattcgag

SEQ ID NO: 17 - DNA, 50 bp, synthetic construct
  source 1..50: mol_type = other DNA
gagcattttttcatgtgccagagcctgtactggaggcccccattgtgcac

SEQ ID NO: 18 - DNA, 50 bp, synthetic construct
  source 1..50: mol_type = other DNA
ctggtctcctcagcttccctatccatataggcacagagaggcagcatttg